European Patent Application EP 4 663 193 A1, published December 17, 2025. Title: PHARMACEUTICAL COMPOSITION FOR PREVENTING OR TREATING AGING MUSCULOSKELETAL DISEASES. Applicant: SEOUL NATIONAL UNIVERSITY R&DB FOUNDATION. The sequence listing filed with the application follows.

SEQUENCE LISTING (9 sequences)

SEQ ID NO: 1 - RNA, 20 nt, synthetic construct
  source 1..20: mol_type = other RNA
ggacgtccgcttcatccatg

SEQ ID NO: 2 - RNA, 20 nt, synthetic construct
  source 1..20: mol_type = other RNA
gcatggatcccaaagcccgg

SEQ ID NO: 3 - RNA, 20 nt, synthetic construct
  source 1..20: mol_type = other RNA
acagccatggctttgatcgg

SEQ ID NO: 4 - RNA, 20 nt, synthetic construct
  source 1..20: mol_type = other RNA
acagccatggctttgatcgg

SEQ ID NO: 5 - RNA, 19 nt, synthetic construct
  source 1..19: mol_type = other RNA
tggcagggctggatacgaa

SEQ ID NO: 6 - RNA, 19 nt, synthetic construct
  source 1..19: mol_type = other RNA
ccgagagagtactgcgcta

SEQ ID NO: 7 - RNA, 19 nt, synthetic construct
  source 1..19: mol_type = other RNA
tggtgaaggtttaccgaga

SEQ ID NO: 8 - RNA, 19 nt, synthetic construct
  source 1..19: mol_type = other RNA
gcttgaaatctctcggata

SEQ ID NO: 9 - RNA, 23 nt, synthetic construct
  source 1..23: mol_type = other RNA
cgcgagcagtacgggcgcgccgg